European Patent Application EP 4 382 121 A1, published June 12, 2024. Title: VACCINES AGAINST PTPRZ1-POSITIVE TUMORS. Applicant: ALTEVAX. The sequence listing filed with the application follows.

SEQUENCE LISTING (16 sequences)

SEQ ID NO: 1 - protein, 9 aa, Synthetic construct
KVFAGIPTV

SEQ ID NO: 2 - protein, 9 aa, Synthetic construct
VLDSHIHAY

SEQ ID NO: 3 - protein, 9 aa, Synthetic construct
AIIDGVESV

SEQ ID NO: 4 - protein, 9 aa, Synthetic construct
MIWEHNVEV

SEQ ID NO: 5 - protein, 10 aa, Synthetic construct
CKVFAGIPTV

SEQ ID NO: 6 - protein, 22 aa, Synthetic construct
CVLDSHIHAYVNALLIPGPAGK

SEQ ID NO: 7 - protein, 10 aa, Synthetic construct
CAIIDGVESV

SEQ ID NO: 8 - protein, 10 aa, Synthetic construct
CMIWEHNVEV

SEQ ID NO: 9 - protein, 10 aa, Synthetic construct
KMIWEHNVEV

SEQ ID NO: 10 - protein, 10 aa, Synthetic construct
PMIWEHNVEV

SEQ ID NO: 11 - protein, 10 aa, Synthetic construct
HMIWEHNVEV

SEQ ID NO: 12 - protein, 11 aa, Synthetic construct
PKMIWEHNVEV

SEQ ID NO: 13 - protein, 11 aa, Synthetic construct
KPMIWEHNVEV

SEQ ID NO: 14 - protein, 11 aa, Synthetic construct
KKKIWEHNVEV

SEQ ID NO: 15 - protein, 9 aa, Synthetic construct
KIWEHNVEV

SEQ ID NO: 16 - DNA, 26 bp, Synthetic construct
  source 1..26: mol_type = other DNA
taaacgttataacgttatgacgtcat